European Patent Application EP 4 796 530 A1, published August 26, 2026. Title: 磺酰脲衍生物及其应用. Applicant: 拜西欧斯（北京）生物技术有限公司. The sequence listing filed with the application follows.

SEQUENCE LISTING (1 sequence)

SEQ ID NO: 1 - DNA, 506 bp, synthetic construct
  source 1..506: mol_type = other DNA
ccatgggccatcatcatcatcatcacggtggctccggcggtagcaaggttgaacaggctgttgaaaccgaaccggaaccggaactgcgtcagcaaaccgagtggcagtctggccagcgttgggagctggcgctgggccgcttttgggactacctgcgttgggtacagactctgtccgaacaggttcaggaagaactgctgtcttcccaggtaacccaggagctgcgcgcactgatggacgagaccatgaaagaactgaaagcctacaagtccgaactggaagaacagctgacgccggttgcggaagaaactcgtgctcgcctgtctaaagaactgcaggctgcgcaggcgcgcctgggcgcggatatggaagatgtttgcggtcgtctggtacagtaccgtggcgaagttcaagctatgctgggccagagcaccgaagaactgcgtgttcgcctggcatcccacctgcgcaaactgcgcaaacgtctgctgcgtgactaactcgag